European Patent Specification EP 3 034 514 B1, published July 17, 2024. Title: ANTIBODY SPECIFICALLY BINDING TO GLP-1R AND FUSION PROTEIN THEREOF WITH GLP-1. Applicant: Gmax Biopharm Co., Ltd. The sequence listing filed with the application follows.

SEQUENCE LISTING (127 sequences)

SEQ ID NO: 1 - protein, 31 aa, Homo sapiens
HAEGTFTSDVSSYLEGQAAKEFIAWLVKGRG

SEQ ID NO: 2 - protein, 31 aa, Homo sapiens
HGEGTFTSDVSSYLEGQAAKEFIAWLVKGRG

SEQ ID NO: 3 - protein, 22 aa, Homo sapiens
HGEGTFTSDVSSYLEGQAAKEF

SEQ ID NO: 4 - protein, 23 aa, Homo sapiens
HGEGTFTSDVSSYLEGQAAKEFI

SEQ ID NO: 5 - protein, 24 aa, Homo sapiens
HGEGTFTSDVSSYLEGQAAKEFIA

SEQ ID NO: 6 - protein, 10 aa, Mouse
GFSLTGYGVN

SEQ ID NO: 7 - protein, 10 aa, Mouse
GFTFSDNGMA

SEQ ID NO: 8 - protein, 10 aa, Mouse
GFTFSDYGMA

SEQ ID NO: 9 - protein, 10 aa, Mouse
GYKFTDYAMY

SEQ ID NO: 10 - protein, 10 aa, Mouse
GYKFTDYAMH

SEQ ID NO: 11 - protein, 12 aa, Mouse
GFSLSTFGMGVG

SEQ ID NO: 12 - protein, 10 aa, Mouse
GFTLSSYGMH

SEQ ID NO: 13 - protein, 17 aa, Mouse
GMIWGGGSTDYNSALKS

SEQ ID NO: 14 - protein, 17 aa, Mouse
FISNLSYRIYYADTVTG

SEQ ID NO: 15 - protein, 17 aa, Mouse
FISNLAYRIYYADTVTG

SEQ ID NO: 16 - protein, 17 aa, Mouse
VISIYYGNTNYNQKFKD

SEQ ID NO: 17 - protein, 17 aa, Mouse
VINIYYGNTSYNQKFKG

SEQ ID NO: 18 - protein, 16 aa, Mouse
HIWWDDDKYYNPALKS

SEQ ID NO: 19 - protein, 17 aa, Mouse
VIWYDGSNKYYADSVKG

SEQ ID NO: 20 - protein, 6 aa, Mouse
GLPGDY

SEQ ID NO: 21 - protein, 11 aa, Mouse
GTMAPNWYFDV

SEQ ID NO: 22 - protein, 11 aa, Mouse
GTTAPNWYFDV

SEQ ID NO: 23 - protein, 9 aa, Mouse
GITTAAFDY

SEQ ID NO: 24 - protein, 9 aa, Mouse
GITMAAFDY

SEQ ID NO: 25 - protein, 9 aa, Mouse
GVTFYAMDH

SEQ ID NO: 26 - protein, 9 aa, Mouse
KGNFAWFTY

SEQ ID NO: 27 - protein, 16 aa, Mouse
GGGSGSYRYYYYGLDV

SEQ ID NO: 28 - protein, 16 aa, Mouse
KSTKSLLNSDGFTYLD

SEQ ID NO: 29 - protein, 10 aa, Mouse
RASSSVTYIH

SEQ ID NO: 30 - protein, 10 aa, Mouse
RASSSVSYMY

SEQ ID NO: 31 - protein, 8 aa, Mouse
QGISNYLN

SEQ ID NO: 32 - protein, 17 aa, Mouse
KSSQSLLNSGNQKNYLA

SEQ ID NO: 33 - protein, 10 aa, Mouse
RASSSVTYIH

SEQ ID NO: 34 - protein, 16 aa, Mouse
RSSKSLLDRNGNTYLY

SEQ ID NO: 35 - protein, 16 aa, Mouse
RSSKSLLHSNGNTYLY

SEQ ID NO: 36 - protein, 17 aa, Mouse
KSSQSLLNSSNQKNYLA

SEQ ID NO: 37 - protein, 11 aa, Mouse
RASQNINNLLA

SEQ ID NO: 38 - protein, 7 aa, Mouse
LVSNRFS

SEQ ID NO: 39 - protein, 7 aa, Mouse
GTSNLAS

SEQ ID NO: 40 - protein, 7 aa, Mouse
ATSNLAS

SEQ ID NO: 41 - protein, 7 aa, Mouse
YTSSLHS

SEQ ID NO: 42 - protein, 7 aa, Mouse
GASTRES

SEQ ID NO: 43 - protein, 7 aa, Mouse
RMSNLAS

SEQ ID NO: 44 - protein, 7 aa, Mouse
FASTRES

SEQ ID NO: 45 - protein, 7 aa, Mouse
TASSLQS

SEQ ID NO: 46 - protein, 9 aa, Mouse
FQSNYLPFT

SEQ ID NO: 47 - protein, 9 aa, Mouse
QQWSSNPPT

SEQ ID NO: 48 - protein, 9 aa, Mouse
QQWTSNPPT

SEQ ID NO: 49 - protein, 9 aa, Mouse
QQYSKLPYT

SEQ ID NO: 50 - protein, 9 aa, Mouse
QNDHSYPFT

SEQ ID NO: 51 - protein, 9 aa, Mouse
MQHLEYPYT

SEQ ID NO: 52 - protein, 9 aa, Mouse
QQHYYTPYT

SEQ ID NO: 53 - protein, 9 aa, Mouse
QQAHRFPPT

SEQ ID NO: 54 - DNA, 342 bp, Mouse
caggtgcaactgaaggagtcaggacctggcctggtggcgccctcacagagcctgtccatcacatgcaccgtctcaggattctcattaaccggctatggtgtaaactgggttcgccagcctccaggaaagggtctggagtggctgggaatgatatggggtggtggaagcacagactataattcagctctcaaatccagactgagcatcagcaaggacaactccaagagccaagttttcttaaaaatgaacagtctgcaaagtgatgacacagccaggtactactgtgccagaggactaccgggggactactggggtcgaggaacctcagtcaccgtctcctca

SEQ ID NO: 55 - protein, 114 aa, Mouse
QVQLKESGPGLVAPSQSLSITCTVSGFSLTGYGVNWVRQPPGKGLEWLGMIWGGGSTDYNSALKSRLSISKDNSKSQVFLKMNSLQSDDTARYYCARGLPGDYWGRGTSVTVSS

SEQ ID NO: 56 - DNA, 360 bp, Mouse
gaggtgaagctggtggagtctgggggcggcatagtgcagcctggagggtcccggaaactctcctgtgcagcctctggattcactttcagtgacaacggaatggcgtgggttcgacaggctccagggaaggggcctgagtgggtagcattcattagtaatttgtcatataggatctactatgcagacactgtgacgggccgattcaccgtctctagagagaatgccaagaacaccctgtacctggaaatgagcagtctgcggtctgaggacacagccttttactactgtgcacggggcactatggctcctaactggtacttcgatgtctggggcgcagggaccacggtcaccgtctcctca

SEQ ID NO: 57 - protein, 120 aa, Mouse
EVKLVESGGGIVQPGGSRKLSCAASGFTFSDNGMAWVRQAPGKGPEWVAFISNLSYRIYYADTVTGRFTVSRENAKNTLYLEMSSLRSEDTAFYYCARGTMAPNWYFDVWGAGTTVTVSS

SEQ ID NO: 58 - DNA, 360 bp, Mouse
gaggtgaaggtggtggagtctgggggaggcttagtgcagcctggagggtcccggaaactctcctgtgcagcctctggattcactttcagtgactacggaatggcgtgggttcgacaggctccagggaaggggcctgagtgggtagcattcattagtaatttggcatatagaatctactatgcagacactgtgacgggccgattcaccatctctagagagaatgccaagaacaccctgtacctggaaatgagcagtctgaggtctgaggacacagccatgtattactgtgcaaggggcactacggctcctaactggtacttcgatgtctggggcgcagggaccacggtcaccgtctcctca

SEQ ID NO: 59 - protein, 120 aa, Mouse
EVKVVESGGGLVQPGGSRKLSCAASGFTFSDYGMAWVRQAPGKGPEWVAFISNLAYRIYYADTVTGRFTISRENAKNTLYLEMSSLRSEDTAMYYCARGTTAPNWYFDVWGAGTTVTVSS

SEQ ID NO: 60 - DNA, 354 bp, Mouse
caggtccagctgcagcagtctgggcctgagctggtgaggcctggggtctcagtgaagatttcctgcaagggttccggctacaaattcactgattatgctatgtactgggtgaagcagagtcatgcaaagagtctagagtggattggagttattagtatttactatggtaatacaaactacaaccagaagtttaaggacaaggccacaatgactgtagacaaatcctccagcacagcctatatggaacttgccagattgacatctgaggattctgccatctattactgtgcaagggggattactacggccgcttttgactactggggccaaggcaccactctcacagtctcctca

SEQ ID NO: 61 - protein, 118 aa, Mouse
QVQLQQSGPELVRPGVSVKISCKGSGYKFTDYAMYWVKQSHAKSLEWIGVISIYYGNTNYNQKFKDKATMTVDKSSSTAYMELARLTSEDSAIYYCARGITTAAFDYWGQGTTLTVSS

SEQ ID NO: 62 - DNA, 354 bp, Mouse
caggtccagctgcagcagtctgggcctgagctggtgaggcctggggtctcagtgaagatttcctgcaagggttccggctacaaattcactgattatgctatgtattgggtgaagcagagtcatgcaaagagtctagagtggattggagttattagtatttattatggtaatacaaactacaaccagaagtttaagggcaaggccacaatgactgtagacaaatcctccaacacagcctatatggaacttgccagattgacatctgaggattctgccatctattactgtgcaagggggattactatggccgcttttgactactggggccaaggcaccactctcacagtctcctca

SEQ ID NO: 63 - protein, 118 aa, Mouse
QVQLQQSGPELVRPGVSVKISCKGSGYKFTDYAMYWVKQSHAKSLEWIGVISIYYGNTNYNQKFKGKATMTVDKSSNTAYMELARLTSEDSAIYYCARGITMAAFDYWGQGTTLTVSS

SEQ ID NO: 64 - DNA, 360 bp, Mouse; identical to SEQ ID NO: 56

SEQ ID NO: 65 - protein, 120 aa, Mouse; identical to SEQ ID NO: 57

SEQ ID NO: 66 - DNA, 354 bp, Mouse
caggtccagctgcagcagtctggggctgagatggtgaggcctggggtctcagtgaagatttcctgcaagggttctggctacaaattcactgattacgctatgcactgggtgaagcagagtcatgcaaagagtctagagtggattggagttattaatatttattatggtaataccagttacaaccagaagttcaagggcaaggccacaatgactattgacagatcctccagcacagcctatatggaacttgccagactgacatctgacgattctgccatctattattgtgcaagaggggttaccttttatgctatggaccactggggtcaaggaacctcagtcaccgtctcctca

SEQ ID NO: 67 - protein, 118 aa, Mouse
QVQLQQSGAEMVRPGVSVKISCKGSGYKFTDYAMHWVKQSHAKSLEWIGVINIYYGNTSYNQKFKGKATMTIDRSSSTAYMELARLTSDDSAIYYCARGVTFYAMDHWGQGTSVTVSS

SEQ ID NO: 68 - DNA, 354 bp, Mouse; identical to SEQ ID NO: 62

SEQ ID NO: 69 - protein, 118 aa, Mouse; identical to SEQ ID NO: 63

SEQ ID NO: 70 - DNA, 357 bp, Mouse
caggttactctgaaagagtctggccctgggatattgcagccctcccagaccctcagtctgacttgttctttctctgggttttcactgagcacttttggtatgggtgtaggctggattcgtcagccttcagggaagggtctggagtggctggcacacatttggtgggatgatgataagtactataacccagccctgaagagtcggctcacaatctccaaggatacctccaaaaaccaggtattcctcaagatcgccaatgtggacactgcagatactgccacatactactgtgctcgaaagggcaacttcgcctggttcacctactggggccaagggactctggtcactgtctctagt

SEQ ID NO: 71 - protein, 119 aa, Mouse
QVTLKESGPGILQPSQTLSLTCSFSGFSLSTFGMGVGWIRQPSGKGLEWLAHIWWDDDKYYNPALKSRLTISKDTSKNQVFLKIANVDTADTATYYCARKGNFAWFTYWGQGTLVTVSS

SEQ ID NO: 72 - DNA, 354 bp, Mouse
caggtccagctgcagcagtctgggcctgagctggtgaggcctggggtctcagtgaagatttcctgcaagggttccggctacaaattcactgattatgctatgcactgggtgaagcaaagtcatgcaaagagtctagagtggattggagttattagtatttactatggtaatacaaactacaaccagaagtttaaggacaaggccacaatgactgtagacaagtcctccagcacagcctatatggaacttgccagattgacatctgaggattctgccatctattactgtgcaagggggattactacggccgcttttgactactggggccaaggcaccactctcacagtctcctca

SEQ ID NO: 73 - protein, 118 aa, Mouse
QVQLQQSGPELVRPGVSVKISCKGSGYKFTDYAMHWVKQSHAKSLEWIGVISIYYGNTNYNQKFKDKATMTVDKSSSTAYMELARLTSEDSAIYYCARGITTAAFDYWGQGTTLTVSS

SEQ ID NO: 74 - DNA, 375 bp, Mouse
caggtgcagctggtggagtctgggggaggcttagtgaagcctggagggtccctgaaactctcctgtgcagcctctggattcaccttaagtagctatggcatgcactgggttcgtcaggctccagagaaggggctggagtgggttgcagtcatatggtatgatggaagtaataaatactatgcagactccgtgaagggccgattcaccatctccagagacaatgccaagaacaccctgttcctgcaaatgaccagtctgaggtctgaggacacggccatgtattactgtgcaagagggggtggttcggggagttatcggtactactactacggtctggacgtctggggcacagggaccacggtcaccgtctctagt

SEQ ID NO: 75 - protein, 125 aa, Mouse
QVQLVESGGGLVKPGGSLKLSCAASGFTLSSYGMHWVRQAPEKGLEWVAVIWYDGSNKYYADSVKGRFTISRDNAKNTLFLQMTSLRSEDTAMYYCARGGGSGSYRYYYYGLDVWGTGTTVTVSS

SEQ ID NO: 76 - DNA, 357 bp, Homo sapiens
caggtcaccctgaaagagtccggccctgccctggtgaagcctacccagaccctgaccctgacatgcaccttcagcggcttcagcctgagcaccttcggcatgggcgtgggctggatcagacagcctcccggcaaggccctggaatggctggcccacatttggtgggacgacgacaagtactacaaccccgccctgaagtcccggctgaccatcagcaaggacaccagcaagaaccaggtggtgctgaccatgaccaacatggaccccgtggacaccgccacctactactgcgcccggaagggcaacttcgcctggttcacctactggggccagggcaccctggtgaccgtctctagt

SEQ ID NO: 77 - protein, 119 aa, Homo sapiens
QVTLKESGPALVKPTQTLTLTCTFSGFSLSTFGMGVGWIRQPPGKALEWLAHIWWDDDKYYNPALKSRLTISKDTSKNQVVLTMTNMDPVDTATYYCARKGNFAWFTYWGQGTLVTVSS

SEQ ID NO: 78 - DNA, 375 bp, Homo sapiens
caggtgcagctggtggagtctgggggaggcgtggtccagcctgggaggtccctgagactctcctgtgcagcgtctggattcaccttaagtagctatggcatgcactgggtccgccaggctccaggcaaggggctggagtgggtggcagtcatatggtatgatggaagtaataaatactatgcagactccgtgaagggccgattcaccatctccagagacaattccaagaacacgctgtatctgcaaatgaacagcctgagagccgaggacacggctgtgtattactgtgcgagagggggtggttcggggagttatcggtactactactacggtctggacgtctggggccaagggaccacggtcaccgtctctagt

SEQ ID NO: 79 - protein, 125 aa, Homo sapiens
QVQLVESGGGVVQPGRSLRLSCAASGFTLSSYGMHWVRQAPGKGLEWVAVIWYDGSNKYYADSVKGRFTISRDNSKNTLYLQMNSLRAEDTAVYYCARGGGSGSYRYYYYGLDVWGQGTTVTVSS

SEQ ID NO: 80 - DNA, 336 bp, Mouse
gatgttgttctgacccaaactccactctctctgcctgtcaatattggagatcaagcctctatctcttgcaagtctactaagagtcttctgaatagtgatggattcacttatttggactggtacctgcagaagccaggccagtctccacagctcctaatatatttggtttctaatcgattttctggagttccagacaggttcagtggcagtgggtcaggaacagatttcacactcaagatcagcagagtggaggctgatgatttgggagtttattattgcttccagagtaactatcttccattcacgttcggctcggggacaaagttggaaataaaa

SEQ ID NO: 81 - protein, 112 aa, Mouse
DVVLTQTPLSLPVNIGDQASISCKSTKSLLNSDGFTYLDWYLQKPGQSPQLLIYLVSNRFSGVPDRFSGSGSGTDFTLKISRVEADDLGVYYCFQSNYLPFTFGSGTKLEIK

SEQ ID NO: 82 - DNA, 318 bp, Mouse
caaattgttctctcccagtctccagcaatcctgtctgcatctccaggggagaaggtcacaatgacttgcagggccagctcaagtgttacttacatacactggtaccagcagaagccaggatcctcccccaaaccctggatttatggcacatccaatctggcttctggagtccctgttcgcttcagtggcagtgggtctgggacctctttctctctcacaatcaccagagtggaggctgaagatgctgccacttattactgccagcagtggagtagtaacccacccacgttcggtactgggaccaagctggagctgaaa

SEQ ID NO: 83 - protein, 106 aa, Mouse
QIVLSQSPAILSASPGEKVTMTCRASSSVTYIHWYQQKPGSSPKPWIYGTSNLASGVPVRFSGSGSGTSFSLTITRVEAEDAATYYCQQWSSNPPTFGTGTKLELK

SEQ ID NO: 84 - DNA, 318 bp, Mouse
caaattgttctctcccagtctccagcaatcctgtctgcatctccaggggagaaggtcacaatgacttgcagggccagctcaagtgtaagttacatgtactggtaccagcagaagccaggatcctcccccaaaccctggatttatgccacatccaacctggcttctggagtccctgctcgcttcagtggcagtgggtctgggacctcttactctctcacaatcagcagagtggaggctgaagatgctgccacttattactgccagcagtggactagtaacccacccacgttcggtgctgggtccaagctggagctgaga

SEQ ID NO: 85 - protein, 106 aa, Mouse
QIVLSQSPAILSASPGEKVTMTCRASSSVSYMYWYQQKPGSSPKPWIYATSNLASGVPARFSGSGSGTSYSLTISRVEAEDAATYYCQQWTSNPPTFGAGSKLELR

SEQ ID NO: 86 - DNA, 324 bp, Mouse
gatatccagatgacacagactacatcctccctgtctgcctctctgggagacagagtcaccatcagttgcagtgcaagtcagggcattagcaattatttaaactggtatcagcagaaaccggatggaactgttaaactcctgatctattacacatcaagtttacactcaggagtcccatcaaggttcagtggcagtgggtctgggacagattattctctcaccatcagcaacctggaacctgaagatgttgccacttactattgtcagcagtatagtaagcttccgtacacgttcggaggggggaccaagctggaaataagacgg

SEQ ID NO: 87 - protein, 108 aa, Mouse
DIQMTQTTSSLSASLGDRVTISCSASQGISNYLNWYQQKPDGTVKLLIYYTSSLHSGVPSRFSGSGSGTDYSLTISNLEPEDVATYYCQQYSKLPYTFGGGTKLEIRR

SEQ ID NO: 88 - DNA, 339 bp, Mouse
gacattgtgatgacacagtctccatcctccctgagtgtgtcagcaggagagaaggtcactatgagctgcaagtccagtcagagtctgttaaacagtggaaatcaaaagaactacttggcctggtaccagcagaaaccagggcagcctcctaaactgttgatctacggggcatccactagggaatctggggtccctgatcgcttcacaggcagtggatctggaactgatttcactcttaccatcagcagtgtgcaggctgaagacctggcagtttattactgtcagaatgatcatagttatccattcacgttcggctcggggacaaagttggaaataaaa

SEQ ID NO: 89 - protein, 113 aa, Mouse
DIVMTQSPSSLSVSAGEKVTMSCKSSQSLLNSGNQKNYLAWYQQKPGQPPKLLIYGASTRESGVPDRFTGSGSGTDFTLTISSVQAEDLAVYYCQNDHSYPFTFGSGTKLEIK

SEQ ID NO: 90 - DNA, 318 bp, Mouse; identical to SEQ ID NO: 82

SEQ ID NO: 91 - protein, 106 aa, Mouse; identical to SEQ ID NO: 83

SEQ ID NO: 92 - DNA, 339 bp, Mouse
gatattgtgatgactcaggctgcaccctctgtacctgtcacttctggagagtcagtatccatctcctgcaggtctagtaagagtctcctggatcgtaatggcaacacttatttatattggttcctgcagaggccaggccagtctcctcagctcctgatatatcggatgtccaaccttgcctcaggagtcccagacaggttcagtggaagtgggtcgggaagtgctttcacactgagaatcagtagagtggaggctgaggatgtgggtgtttattactgtatgcaacatctagaatatccgtacacgttcggaggggggaccaagctggaaataaaacgg

SEQ ID NO: 93 - protein, 113 aa, Mouse
DIVMTQAAPSVPVTSGESVSISCRSSKSLLDRNGNTYLYWFLQRPGQSPQLLIYRMSNLASGVPDRFSGSGSGSAFTLRISRVEAEDVGVYYCMQHLEYPYTFGGGTKLEIKR

SEQ ID NO: 94 - DNA, 339 bp, Mouse
gatattgtgatgactcaggctgcaccctctgtacctgtcactcctggagcgtcagtatccatctcctgcaggtctagtaagagtctcctgcatagtaatggcaacacttatttgtattggttcctgcagaggccaggccagtctcctcacctcctgatatatcggatgtccaaccttgcctcgggagtcccagacaggttcagtggcagtgggtcaggaactgctttcacactgagaatcagtagagtggaggctgaggatgtgggtgtttattactgtatgcaacatctagaatatccgtacacgttcggaggggggaccaagctggaaataaaacgg

SEQ ID NO: 95 - protein, 113 aa, Mouse
DIVMTQAAPSVPVTPGASVSISCRSSKSLLHSNGNTYLYWFLQRPGQSPHLLIYRMSNLASGVPDRFSGSGSGTAFTLRISRVEAEDVGVYYCMQHLEYPYTFGGGTKLEIKR

SEQ ID NO: 96 - DNA, 339 bp, Mouse
gacattgtgatgacacagtctccatcctccctggctatgtcagtaggacagaaggtcactatgagctgcaagtccagtcagagccttttaaatagtagcaatcaaaagaactatttggcctggtaccagcagaaaccaggacagtctcctaaacttctgatatactttgcatccactagggaatctggggtccctgatcgcttcataggcagtggatctgggacagatttcactcttaccatcagcagtgtgcaggctgaagacctggcagattacttctgtcagcaacattattacactccttacacgttcggaggggggaccaagctggaaataaaa

SEQ ID NO: 97 - protein, 113 aa, Mouse
DIVMTQSPSSLAMSVGQKVTMSCKSSQSLLNSSNQKNYLAWYQQKPGQSPKLLIYFASTRESGVPDRFIGSGSGTDFTLTISSVQAEDLADYFCQQHYYTPYTFGGGTKLEIK

SEQ ID NO: 98 - DNA, 339 bp, Mouse
gatattgtgatgactcaggctgcaccctctgtacctgtcactcctggagagtcagtatccatctcctgcaggtctagtaagagtctcctgcatagtaatggcaacacttacttgtattggttcctgcagaggccaggccagtctcctcagctcctgatttatcggatgtccaaccttgcctcaggagtcccagacaggttcagtggcagtgggtcaggaactgctttcacactgagaatcagtagagtggaggctgaggatgtgggtatttattactgtatgcaacatctagaatatccgtacacgttcggaggggggaccaagctggaaataaaacgg

SEQ ID NO: 99 - protein, 113 aa, Mouse
DIVMTQAAPSVPVTPGESVSISCRSSKSLLHSNGNTYLYWFLQRPGQSPQLLIYRMSNLASGVPDRFSGSGSGTAFTLRISRVEAEDVGIYYCMQHLEYPYTFGGGTKLEIKR

SEQ ID NO: 100 - DNA, 324 bp, Mouse
gccatcaagatgacccagtctccatcttccatgtatgcatctctaggagagagagtcactatcacttgccgggcgagtcaaaatattaacaacttattagcctggttccagcagaaaccagggaaatctcctaagaccctgatctatactgcatccagtttgcaaagtggggtcccatcaaggttcagtggcagtggatctgggcaagattattctctcaccatcagcagcctggagtatgaagatatgggaatttattattgtcaacaggctcatagattccctccgacgttcggtggaggcaccaagctggaaatcagacgt

SEQ ID NO: 101 - protein, 108 aa, Mouse
AIKMTQSPSSMYASLGERVTITCRASQNINNLLAWFQQKPGKSPKTLIYTASSLQSGVPSRFSGSGSGQDYSLTISSLEYEDMGIYYCQQAHRFPPTFGGGTKLEIRR

SEQ ID NO: 102 - DNA, 339 bp, Homo sapiens
gacatcgtgatgacccagagccccgatagcctggccgtgtctctgggcgagcgggccaccatcaactgcaagagcagccagagcctgctgaacagcagcaaccagaagaactacctggcctggtatcagcagaagcccggccagccccccaagctgctgatctacttcgccagcaccagagaaagcggcgtgcccgacagattttctggcagcggcagcggcaccgactttaccctgacaatcagctctctgcaggccgaggacgtggccgtgtacttctgccagcagcactactacaccccctacaccttcggcggaggcaccaaggtggagatcaag

SEQ ID NO: 103 - protein, 113 aa, Homo sapiens
DIVMTQSPDSLAVSLGERATINCKSSQSLLNSSNQKNYLAWYQQKPGQPPKLLIYFASTRESGVPDRFSGSGSGTDFTLTISSLQAEDVAVYFCQQHYYTPYTFGGGTKVEIK

SEQ ID NO: 104 - DNA, 324 bp, Homo sapiens
gccatccagatgacccagtctccatcttccgtgtctgcttctataggagacagagtcaccatcacttgtcgggcgagtcaaaatattaacaacttattagcctggtatcagcagaaaccagggaaagcccccaaactcctgatctatactgcatccagtttgcaaagtgaggtcccatcaaggttcagcggcagtgggtctgggacagatttcactctcaccatcagcagcctgcagcctgaagattttgcaatttactgttgccaacaggctcatagattccctccgacgttcggccaagggaccaaggtggaaatcagacgt

SEQ ID NO: 105 - protein, 108 aa, Homo sapiens
AIQMTQSPSSVSASIGDRVTITCRASQNINNLLAWYQQKPGKAPKLLIYTASSLQSEVPSRFSGSGSGTDFTLTISSLQPEDFAIYCCQQAHRFPPTFGQGTKVEIRR

SEQ ID NO: 106 - protein, 106 aa, Mouse
ADAAPTVSIFPPSSEQLTSGGASVVCFLNNFYPKDINVKWKIDGSERQNGVLNSWTDQDSKDSTYSMSSTLTLTKDEYERHNSYTCEATHKTSTSPIVKSFNRNEC

SEQ ID NO: 107 - protein, 105 aa, Mouse
GQPKSTPTLTVFPPSSEELKENKATLVCLISNFSPSGVTVAWKANGTPITQGVDTSNPTKEGNKFMASSFLHLTSDQWRSHNSFTCQVTHEGDTVEKSLSPAECL

SEQ ID NO: 108 - protein, 325 aa, Mouse
AKTTAPSVYPLAPVCGDTTGSSVTLGCLVKGYFPEPVTLTWNSGSLSSGVHTFPAVLQSDLYTLSSSVTVPSSTWPSETVTCNVAHPASSTKVDKKIVPRDCGCKPCICTVPEVSSVFIFPPKPKDVLTITLTPKVTCVVVDISKDDPEVQFSWFVDDVEVHTAQTQPREEQFNSTFRSVSELPIMHQDWLNGKEFKCRVNSAAFPAPIEKTISKTKGRPKAPQVYTIPPPKEQMAKDKVSLTCMITDFFPEDITVEWQWNGQPAENYKNTQPIMDTDGSYFVYSKLNVQKSNWEAGNTFTCSVLHEGLHNHHTEKSLSHSPGKG

SEQ ID NO: 109 - protein, 326 aa, Homo sapiens
ASTKGPSVFPLAPCSRSTSESTAALGCLVKDYFPEPVTVSWNSGALTSGVHTFPAVLQSSGLYSLSSVVTVPSSNFGTQTYTCNVDHKPSNTKVDKTVERKCCVECPPCPAPPVAGPSVFLFPPKPKDTLMISRTPEVTCVVVDVSHEDPEVQFNWYVDGVEVHNAKTKPREEQFNSTFRVVSVLTVVHQDWLNGKEYKCKVSNKGLPAPIEKTISKTKGQPREPQVYTLPPSREEMTKNQVSLTCLVKGFYPSDIAVEWESNGQPENNYKTTPPMLDSDGSFFLYSKLTVDKSRWQQGNVFSCSVMHEALHNHYTQKSLSLSPGK

SEQ ID NO: 110 - protein, 16 aa, Artificial sequence
GGGSGGGSGGGSGGGS

SEQ ID NO: 111 - protein, 23 aa, Artificial sequence
GSGSATGGSGSGASSGSGSATGS

SEQ ID NO: 112 - protein, 12 aa, Artificial sequence
KDIDRKCCVECP

SEQ ID NO: 113 - DNA, 3123 bp, Homo sapiens
atcagtctccgcacgcggttccgcaggtggcagcgatggcccagtcctgaactccccgccatggccggcgcccccggcccgctgcgccttgcgctgctgctgctcgggatggtgggcagggccggcccccgcccccagggtgccactgtgtccctctgggagacggtgcagaaatggcgagaataccgacgccagtgccagcgctccctgactgaggatccacctcctgccacagacttgttctgcaaccggaccttcgatgaatacgcctgctggccagatggggagccaggctcgttcgtgaatgtcagctgcccctggtacctgccctgggccagcagtgtgccgcagggccacgtgtaccggttctgcacagctgaaggcctctggctgcagaaggacaactccagcctgccctggagggacttgtcggagtgcgaggagtccaagcgaggggaaagaagctccccggaggagcagctcctgttcctctacatcatctacacggtgggctacgcactctccttctctgctctggttatcgcctctgcgatcctcctcggcttcagacacctgcactgcaccaggaactacatccacctgaacctgtttgcatccttcatcctgcgagcattgtccgtcttcatcaaggacgcagccctgaagtggatgtatagcacagccgcccagcagcaccagtgggatgggctcctctcctaccaggactctctgagctgccgcctggtgtttctgctcatgcagtactgtgtggcggccaattactactggctcttggtggagggcgtgtacctgtacacactgctggccttctcggtcttatctgagcaatggatcttcaggctctacgtgagcataggctggggtgttcccctgctgtttgttgtcccctggggcattgtcaagtacctctatgaggacgagggctgctggaccaggaactccaacatgaactactggctcattatccggctgcccattctctttgccattggggtgaacttcctcatctttgttcgggtcatctgcatcgtggtatccaaactgaaggccaatctcatgtgcaagacagacatcaaatgcagacttgccaagtccacgctgacactcatccccctgctggggactcatgaggtcatctttgcctttgtgatggacgagcacgcccgggggaccctgcgcttcatcaagctgtttacagagctctccttcacctccttccaggggctgatggtggccatattatactgctttgtcaacaatgaggtccagctggaatttcggaagagctgggagcgctggcggcttgagcacttgcacatccagagggacagcagcatgaagcccctcaagtgtcccaccagcagcctgagcagtggagccacggcgggcagcagcatgtacacagccacttgccaggcctcctgcagctgagactccagcgcctgccctccctggggtccttgctgcaggccgggtggccaatccaggtgggagagacactcccagggacaagggaaggaagggacacacacacacacacacacacacacacacacacacacatacatcctgctttccctccccaaacccatcagacaggtaaatgggcagtgcctcctgggaccatggacacattttctcctaggagaagcagcctcctaatttgatcacagtggcgagaggagaggaaaaacgatcgctgtgaaaatgaggaggattgcttcttgtgaaaccacaggcccttggggttcccccagacagagccgcaaatcaaccccagactcaaactcaaggtcaacggcttattagtgaaactggggcttgcaagaggaggtggttctgaaagtggctcttctaacctcagccaaacacagagcgggagtgacgggagcctcctctgcttgcatcacttggggtcaccaccctcccctgtcttctctcaaagggaagctgtttgtgtgtctgggttgcttatttccctcatcttgccccctcatctcactgcccagtttctttttgaggggctttgtttgggccactgccagcagctgtttctggaaatggctgtaggtggtgttgagaaagaatgagcattgagacggtgctcgcttctcctccaggtatttgagttgttttggtgcctgcctctgccatgcccagagaatcagggcaggcttgccaccggggaacccagccctggggtatgagctgccaagtctattttaaagacgctcaagaatcctctggggttcatctagggacacgttaggaatgtccagactgtgggtgtagattacctgccacttccaggagcccagagggccaagagagacattgcctccacctctccttggaaatactttatctgtgaccacacgctgtctcttgagaatttggatacactctctagctttaggggaccatgaagagactctcttagggaaaccaatagtccccatcagcaccatggaggcaggctccccctgcctttgaaattcccccacttgggagcttgtatatacttcactcacttttctttattgctgtgaatagtctgtgtgcacaatgggcaattctgacttctcccatctagtggaaatgagcgaaatcatggttgtagtgatgttgtttgggagagtgcagtagtaattgatttgacccactcacacttggagctaattaaggtttgccctgcctgcagcctcccccacaaataatgaacagcagaaagactggacggggaaacctatcaatcctgcccccagccatggtgaggaagccccaagccatggtgacacacagcagcactgcagatagccagacacatggctatcctagagaggctggcaaggagttcgtggctgcaaaagaagtttctggagcaagagagagctcgctcttgggagtcaggacctccggggagagcagagggttccgacggattcctttatgagtcagtctctctctcccttttaaatggtgggaaccctccccaaaacctttccccagacacattctcctgtgcccctcagagaggcatgtgatgtgcaaggaaaataataggatataaaacacatcaagtagaaaatttcttatacttca

SEQ ID NO: 114 - protein, 463 aa, Homo sapiens [sequence omitted]

SEQ ID NO: 115 - DNA, 20 bp, Artificial sequence
tttggrgggaagatgaagac

SEQ ID NO: 116 - DNA, 21 bp, Artificial sequence
ttaacactctcccctgttgaa

SEQ ID NO: 117 - DNA, 21 bp, Artificial sequence
ttaacactcattcctgttgaa

SEQ ID NO: 118 - DNA, 21 bp, Artificial sequence
tggacagggatccagagttcc

SEQ ID NO: 119 - DNA, 21 bp, Artificial sequence
tggacagggctccatagttcc

SEQ ID NO: 120 - DNA, 20 bp, Artificial sequence
actcgtccttggtcaacgtg

SEQ ID NO: 121 - DNA, 23 bp, Artificial sequence
ccaccatggactttgggctgagc

SEQ ID NO: 122 - DNA, 20 bp, Artificial sequence
agagccggtggcagagccag

SEQ ID NO: 123 - DNA, 43 bp, Artificial sequence
ctggctctgccaccggctctgccatccagatgacccagtctcc

SEQ ID NO: 124 - DNA, 22 bp, Artificial sequence
acactctcccctgttgaagctc

SEQ ID NO: 125 - DNA, 31 bp, Artificial sequence
ccggctagccaccatggactttgggctgagc

SEQ ID NO: 126 - DNA, 36 bp, Artificial sequence
agtgcggccgctcaacactctcccctgttgaagctc

SEQ ID NO: 127 - protein, 39 aa, Heloderma suspectum
HGEGTFTSDLSKQMEEEAVRLFIEWLKNGGPSSGAPPPS